European Patent Application EP 4 803 098 A1, published September 9, 2026. Title: GIPR 阻断型抗体及其抗体偶联物. Applicant: 山东博安生物技术股份有限公司. Application WO. The sequence listing filed with the application follows.

SEQUENCE LISTING (53 sequences)

SEQ ID NO: 1 - protein, 107 aa, synthetic construct
DIQMTQSPSSLSASVGDRVTITCRASQGISNYLAWFQQKPGKAPKSLIYAASSLQSGVPSKFSGSGSGTDFTLTISSLQPEDFATYYCQQYNSYPITFGQGTRLEIK

SEQ ID NO: 2 - protein, 121 aa, synthetic construct
EVQLVQSGAEVKKPGSSVKVSCKASGGTFSTFSSYAISWVRQAPGQGLEWMGRIIPILGIGNNAQKFQGRVTITADKSTSTAYMELSSLRSEDTAVYYCAREKDWGHFDYWGQGTLVTVSS

SEQ ID NO: 3 - protein, 6 aa, synthetic construct
QGISNY

SEQ ID NO: 4 - skipped

SEQ ID NO: 5 - protein, 9 aa, synthetic construct
QQYNSYPIT

SEQ ID NO: 6 - protein, 11 aa, synthetic construct
GGTFSTFSSYA

SEQ ID NO: 7 - protein, 8 aa, synthetic construct
IIPILGIG

SEQ ID NO: 8 - protein, 11 aa, synthetic construct
AREKDWGHFDY

SEQ ID NO: 9 - protein, 107 aa, synthetic construct
DIQMTQSPSSLSASVGDRVTITCRASQGISNYLAWFQQKPGKAPKSLIYAASSLQSGVPSRFSGSGSGTDFTLTISNLQPEDFATYYCLQYYDYPLTFGGGTKLEIK

SEQ ID NO: 10 - protein, 118 aa, synthetic construct
EVQLVQSGAEVKKPGSSVKVSCKASGGTFNNYAISWVRQAPGQGLEWMGRIIPFLDIASNAQKFQGKVTITADKSTSTAYMELSSLRSEDTAVYYCAREVDWGWFDSWGQGTLVTVSS

SEQ ID NO: 11 - protein, 6 aa, synthetic construct
QGISNY

SEQ ID NO: 12 - skipped

SEQ ID NO: 13 - protein, 9 aa, synthetic construct
LQYYDYPLT

SEQ ID NO: 14 - protein, 8 aa, synthetic construct
GGTFNNYA

SEQ ID NO: 15 - protein, 8 aa, synthetic construct
IIPFLDIA

SEQ ID NO: 16 - protein, 11 aa, synthetic construct
AREVDWGWFDS

SEQ ID NO: 17 - protein, 107 aa, synthetic construct
DIQLTQSPSSLSASVGDRVTITCRASQTISRFLNWYQQKPGKAPELLIYVASSLQSGVPSRFSGSGSGTDFTLTISSLQPEDFATYYCQQSYSTLISFGQGTKLEIT

SEQ ID NO: 18 - protein, 121 aa, synthetic construct
QVQLVESGGGVVQPGRSLRLSCTASGFTFSSYGIHWVRQAPGKGLEWVAVIWYDGSNKFHADSVKGRFTISRDNSKNTLYLQMNSLRAEDSAMYFCARGKVAGMPEAFEIWGQGTKVTVSS

SEQ ID NO: 19 - protein, 6 aa, synthetic construct
QTISRF

SEQ ID NO: 20 - skipped

SEQ ID NO: 21 - protein, 9 aa, synthetic construct
QQSYSTLIS

SEQ ID NO: 22 - protein, 8 aa, synthetic construct
GFTFSSYG

SEQ ID NO: 23 - protein, 8 aa, synthetic construct
IWYDGSNK

SEQ ID NO: 24 - protein, 14 aa, synthetic construct
ARGKVAGMPEAFEI

SEQ ID NO: 25 - protein, 107 aa, synthetic construct
EIVMTQSPATLSVSPGERATLSCRASQSVSSNLAWYQQKPGQAPRLLIYGAATRATGIPARVSGSGSGTEFTLTISSLQSEDFAVYYCQQYNNWPLTFGGGTKVEIK

SEQ ID NO: 26 - protein, 120 aa, synthetic construct
QVQLVESGGGVVQPGRSLRLSCAASGFTFSNYGMHWVRQAPGEGLEWVAAIWFDASDKYYADAVKGRFTISRDNSKNTLYLQMNSLRAEDTAVYYCARDQAIFGVVPDYWGQGTLVTVSS

SEQ ID NO: 27 - protein, 6 aa, synthetic construct
QSVSSN

SEQ ID NO: 28 - skipped

SEQ ID NO: 29 - protein, 9 aa, synthetic construct
QQYNNWPLT

SEQ ID NO: 30 - protein, 8 aa, synthetic construct
GFTFSNYG

SEQ ID NO: 31 - protein, 8 aa, synthetic construct
IWFDASDK

SEQ ID NO: 32 - protein, 13 aa, synthetic construct
ARDQAIFGVVPDY

SEQ ID NO: 33 - protein, 330 aa, synthetic construct
ASTKGPSVFPLAPSSKSTSGGTAALGCLVKDYFPEPVTVSWNSGALTSGVHTFPAVLQSSGLYSLSSVVTVPSSSLGTQTYICNVNHKPSNTKVDKKVEPKSCDKTHTCPPCPAPEAAGGPSVFLFPPKPKDTLMISRTPEVTCVVVDVSHEDPEVKFNWYVDGVEVHNAKTKPREEQYNSTYRVVSVLTVLHQDWLNGKEYKCKVSNKALAAPIEKTISKAKGQPREPQVYTLPPSRDELTKNQVSLTCLVKGFYPSDIAVEWESNGQPENNYKTTPPVLDSDGSFFLYSKLTVDKSRWQQGNVFSCSVMHEALHNHYTQKSLSLSPGK

SEQ ID NO: 34 - protein, 107 aa, synthetic construct [sequence omitted]

SEQ ID NO: 35 - protein, 47 aa, synthetic construct
HXEGTFTSDVSSYLEEQAAKEFIAWLVKGGGGGGGSGGGGSGGGGSK

SEQ ID NO: 36 - protein, 47 aa, synthetic construct
HXEGTFTSDYSSYLEEQAAKEFIAWLVKGGGGGGGSGGGGSGGGGSK

SEQ ID NO: 37 - protein, 47 aa, synthetic construct
HXEGTFTSDVSSYLEGQAAKEFIAWLVKGRGGGGGSGGGGSGGGGSK

SEQ ID NO: 38 - protein, 107 aa, synthetic construct
DIVMTQSPATLSVSPGERATLSCRASQSVSSNLAWYQQKPGQAPRLLIYGASTRATGIPARFSGSGSGTEFTLTISSLQSEDFAVYYCQQYNNWPLTFGGGTKVEIK

SEQ ID NO: 39 - protein, 119 aa, synthetic construct
EVQLVQSGAEVKKPGSSVKVSCKASGGTFSGYPINWVRQAPGQGLEWMGRIIPIPGIPNYAQKFQDRVTITADKFANTAYMELSSLRSEDTAVYYCARDPLGPYVFDIWGQGTMVTVSS

SEQ ID NO: 40 - protein, 6 aa, synthetic construct
QSVSSN

SEQ ID NO: 41 - skipped

SEQ ID NO: 42 - protein, 9 aa, synthetic construct
QQYNNWPLT

SEQ ID NO: 43 - protein, 8 aa, synthetic construct
GGTFSGYP

SEQ ID NO: 44 - protein, 8 aa, synthetic construct
IIPIPGIP

SEQ ID NO: 45 - protein, 12 aa, synthetic construct
ARDPLGPYVFDI

SEQ ID NO: 46 - protein, 106 aa, synthetic construct
IQMTQSPSSLSASVGDRVTITCRASQGISSYLAWYQQKPGKAPKLLIYAASTLQSGVPSRFSGSGSGTDFTLTISSLQPEDFATYYCQQLNSYPLTFGGGTKVEIK

SEQ ID NO: 47 - protein, 118 aa, synthetic construct
EVQLVQSGAEVKKPGSSVKVSCKASGGTFNNYAISWVRQAPGQGLEWMGRIIPFLDIASYAQKFQGKVTITADKSTSTAYMELSSLRSEDTAVYYCAREVDWGWFDSWGQGTLVTVSS

SEQ ID NO: 48 - protein, 6 aa, synthetic construct
QGISSY

SEQ ID NO: 49 - skipped

SEQ ID NO: 50 - protein, 9 aa, synthetic construct
QQLNSYPLT

SEQ ID NO: 51 - protein, 8 aa, synthetic construct
GGTFNNYA

SEQ ID NO: 52 - protein, 8 aa, synthetic construct
IIPFLDIA

SEQ ID NO: 53 - protein, 11 aa, synthetic construct
AREVDWGWFDS